European Patent Application EP 4 461 822 A1, published November 13, 2024. Title: 유전자 편집 과정에서 발생 가능한 오프 타겟을 예측하는 방법. Applicant: 주식회사 툴젠. Application KR. The sequence listing filed with the application follows.

SEQUENCE LISTING (383 sequences)

SEQ ID NO: 1 - protein, 7 aa, synthetic construct
PKKKRKV

SEQ ID NO: 2 - protein, 16 aa, synthetic construct
KRPAATKKAGQAKKKK

SEQ ID NO: 3 - protein, 9 aa, synthetic construct
PAAKRVKLD

SEQ ID NO: 4 - protein, 11 aa, synthetic construct
RQRRNELKRSP

SEQ ID NO: 5 - protein, 38 aa, synthetic construct
NQSSNFGPMKGGNFGGRSSGPYGGGGQYFAKPRNQGGY

SEQ ID NO: 6 - protein, 42 aa, synthetic construct
RMRIZFKNKGKDTAELRRRRVEVSVELRKAKKDEQILKRRNV

SEQ ID NO: 7 - protein, 8 aa, synthetic construct
VSRKRPRP

SEQ ID NO: 8 - protein, 8 aa, synthetic construct
PPKKARED

SEQ ID NO: 9 - protein, 8 aa, synthetic construct
POPKKKPL

SEQ ID NO: 10 - protein, 12 aa, synthetic construct
SALIKKKKKMAP

SEQ ID NO: 11 - protein, 5 aa, synthetic construct
DRLRR

SEQ ID NO: 12 - protein, 7 aa, synthetic construct
PKQKKRK

SEQ ID NO: 13 - protein, 10 aa, synthetic construct
RKLKKKIKKL

SEQ ID NO: 14 - protein, 10 aa, synthetic construct
REKKKFLKRR

SEQ ID NO: 15 - protein, 20 aa, synthetic construct
KRKGDEVDGVDEVAKKKSKK

SEQ ID NO: 16 - protein, 17 aa, synthetic construct
RKCLQAGMNLEARKTKK

SEQ ID NO: 17 - protein, 30 aa, synthetic construct
MDSLLMNRRKFLYQFKNVRWAKGRRETYLC

SEQ ID NO: 18 - skipped

SEQ ID NO: 19 - protein, 8 aa, synthetic construct
NNNNRYAC

SEQ ID NO: 20 - protein, 7 aa, synthetic construct
NNAGAAW

SEQ ID NO: 21 - protein, 8 aa, synthetic construct
NNNNGATT

SEQ ID NO: 22 - protein, 6 aa, synthetic construct
NNGRRT

SEQ ID NO: 23 - skipped

SEQ ID NO: 24 - protein, 8 aa, synthetic construct
NNNVRYAC

SEQ ID NO: 25 - DNA, 19 bp, synthetic construct
  source 1..19: mol_type = other DNA
aggtgggaaactgaggctt

SEQ ID NO: 26 - DNA, 19 bp, synthetic construct
  source 1..19: mol_type = other DNA
acatgcatatgtatgtgtg

SEQ ID NO: 27 - DNA, 20 bp, synthetic construct
  source 1..20: mol_type = other DNA
gacatgcatatgtatgtgtg

SEQ ID NO: 28 - DNA, 20 bp, synthetic construct
  source 1..20: mol_type = other DNA
gaggtgggaaactgaggctt

SEQ ID NO: 29 - RNA, 102 nt, synthetic construct
  source 1..102: mol_type = other RNA
gaggtgggaaactgaggcttgttttagagctagaaatagcaagttaaaataaggctagtccgttatcaacttgaaaaagtggcaccgagtcggtgctttttt

SEQ ID NO: 30 - RNA, 20 nt, synthetic construct
  source 1..20: mol_type = other RNA
gaggtgggaaactgaggctt

SEQ ID NO: 31 - RNA, 102 nt, synthetic construct
  source 1..102: mol_type = other RNA
gacatgcatatgtatgtgtggttttagagctagaaatagcaagttaaaataaggctagtccgttatcaacttgaaaaagtggcaccgagtcggtgctttttt

SEQ ID NO: 32 - RNA, 20 nt, synthetic construct
  source 1..20: mol_type = other RNA
gacatgcatatgtatgtgtg

SEQ ID NO: 33 - RNA, 102 nt, synthetic construct
  source 1..102: mol_type = other RNA
ggaatcccttctgcagcaccgttttagagctagaaatagcaagttaaaataaggctagtccgttatcaacttgaaaaagtggcaccgagtcggtgctttttt

SEQ ID NO: 34 - RNA, 20 nt, synthetic construct
  source 1..20: mol_type = other RNA
ggaatcccttctgcagcacc

SEQ ID NO: 35 - DNA, 19 bp, synthetic construct
  source 1..19: mol_type = other DNA
gaatcccttctgcagcacc

SEQ ID NO: 36 - RNA, 102 nt, synthetic construct
  source 1..102: mol_type = other RNA
gggtggggggagtttgctccgttttagagctagaaatagcaagttaaaataaggctagtccgttatcaacttgaaaaagtggcaccgagtcggtgctttttt

SEQ ID NO: 37 - RNA, 20 nt, synthetic construct
  source 1..20: mol_type = other RNA
gggtggggggagtttgctcc

SEQ ID NO: 38 - DNA, 19 bp, synthetic construct
  source 1..19: mol_type = other DNA
ggtggggggagtttgctcc

SEQ ID NO: 39 - RNA, 102 nt, synthetic construct
  source 1..102: mol_type = other RNA
gttgccccacagggcagtaagttttagagctagaaatagcaagttaaaataaggctagtccgttatcaacttgaaaaagtggcaccgagtcggtgctttttt

SEQ ID NO: 40 - RNA, 20 nt, synthetic construct
  source 1..20: mol_type = other RNA
gttgccccacagggcagtaa

SEQ ID NO: 41 - DNA, 19 bp, synthetic construct
  source 1..19: mol_type = other DNA
ttgccccacagggcagtaa

SEQ ID NO: 42 - protein, 1368 aa, synthetic construct [sequence omitted]

SEQ ID NO: 43 - DNA, 4104 bp, synthetic construct
  source 1..4104: mol_type = other DNA
atggacaagaagtacagcatcggcctggacatcggtaccaacagcgtgggctgggccgtgatcaccgacgagtacaaggtgcccagcaagaagttcaaggtgctgggcaacaccgaccgccacagcatcaagaagaacctgatcggcgccctgctgttcgacagcggcgagaccgccgaggccacccgcctgaagcgcaccgcccgccgccgctacacccgccgcaagaaccgcatctgctacctgcaggagatcttcagcaacgagatggccaaggtggacgacagcttcttccaccgcctggaggagagcttcctggtggaggaggacaagaagcacgagcgccaccccatcttcggcaacatcgtggacgaggtggcctaccacgagaagtaccccaccatctaccacctgcgcaagaagctggtggacagcaccgacaaggccgacctgcgcctgatctacctggccctggcccacatgatcaagttccgcggccacttcctgatcgagggcgacctgaaccccgacaacagcgacgtggacaagctgttcatccagctggtgcagacctacaaccagctgttcgaggagaaccccatcaacgccagcggcgtggacgccaaggccatcctgagcgcccgcctgagcaagagccgccgcctggagaacctgatcgcccagctgcccggcgagaagaagaacggcctgttcggcaacctgatcgccctgagcctgggcctgacccccaacttcaagagcaacttcgacctggccgaggacgccaagctgcagctgagcaaggacacctacgacgacgacctggacaacctgctggcccagatcggcgaccagtacgccgacctgttcctggccgccaagaacctgagcgacgccatcctgctgagcgacatcctgcgcgtgaacaccgagatcaccaaggcccccctgagcgccagcatgatcaagcgctacgacgagcaccaccaggacctgaccctgctgaaggccctggtgcgccagcagctgcccgagaagtacaaggagatcttcttcgaccagagcaagaacggctacgccggctacatcgacggcggcgccagccaggaggagttctacaagttcatcaagcccatcctggagaagatggacggcaccgaggagctgctggtgaagctgaaccgcgaggacctgctgcgcaagcagcgcaccttcgacaacggcagcatcccccaccagatccacctgggcgagctgcacgccatcctgcgccgccaggaggacttctaccccttcctgaaggacaaccgcgagaagatcgagaagatcctgaccttccgcatcccctactacgtgggccccctggcccgcggcaacagccgcttcgcctggatgacccgcaagagcgaggagaccatcaccccctggaacttcgaggaggtggtggacaagggcgccagcgcccagagcttcatcgagcgcatgaccaacttcgacaagaacctgcccaacgagaaggtgctgcccaagcacagcctgctgtacgagtacttcaccgtgtacaacgagctgaccaaggtgaagtacgtgaccgagggcatgcgcaagcccgccttcctgagcggcgagcagaagaaggccatcgtggacctgctgttcaagaccaaccgcaaggtgaccgtgaagcagctgaaggaggactacttcaagaagatcgagtgcttcgacagcgtggagatcagcggcgtggaggaccgcttcaacgccagcctgggcacctaccacgacctgctgaagatcatcaaggacaaggacttcctggacaacgaggagaacgaggacatcctggaggacatcgtgctgaccctgaccctgttcgaggaccgcgagatgatcgaggagcgcctgaagacctacgcccacctgttcgacgacaaggtgatgaagcagctgaagcgccgccgctacaccggctggggccgcctgagccgcaagcttatcaacggcatccgcgacaagcagagcggcaagaccatcctggacttcctgaagagcgacggcttcgccaaccgcaacttcatgcagctgatccacgacgacagcctgaccttcaaggaggacatccagaaggcccaggtgagcggccagggcgacagcctgcacgagcacatcgccaacctggccggcagccccgccatcaagaagggcatcctgcagaccgtgaaggtggtggacgagctggtgaaggtgatgggccgccacaagcccgagaacatcgtgatcgagatggcccgcgagaaccagaccacccagaagggccagaagaacagccgcgagcgcatgaagcgcatcgaggagggcatcaaggagctgggcagccagatcctgaaggagcaccccgtggagaacacccagctgcagaacgagaagctgtacctgtactacctgcagaacggccgcgacatgtacgtggaccaggagctggacatcaaccgcctgagcgactacgacgtggaccacatcgtgccccagagcttcctgaaggacgacagcatcgacaacaaggtgctgacccgcagcgacaagaaccgcggcaagagcgacaacgtgcccagcgaggaggtggtgaagaagatgaagaactactggcgccagctgctgaacgccaagctgatcacccagcgcaagttcgacaacctgaccaaggccgagcgcggcggcctgagcgagctggacaaggccggcttcatcaagcgccagctggtggagacccgccagatcaccaagcacgtggcccagatcctggacagccgcatgaacaccaagtacgacgagaacgacaagctgatccgcgaggtgaaggtgatcaccctgaagagcaagctggtgagcgacttccgcaaggacttccagttctacaaggtgcgcgagatcaacaactaccaccacgcccacgacgcctacctgaacgccgtggtgggcaccgccctgatcaagaagtaccccaagctggagagcgagttcgtgtacggcgactacaaggtgtacgacgtgcgcaagatgatcgccaagagcgagcaggagatcggcaaggccaccgccaagtacttcttctacagcaacatcatgaacttcttcaagaccgagatcaccctggccaacggcgagatccgcaagcgccccctgatcgagaccaacggcgagaccggcgagatcgtgtgggacaagggccgcgacttcgccaccgtgcgcaaggtgctgagcatgccccaggtgaacatcgtgaagaagaccgaggtgcagaccggcggcttcagcaaggagagcatcctgcccaagcgcaacagcgacaagctgatcgcccgcaagaaggactgggaccccaagaagtacggcggcttcgacagccccaccgtggcctacagcgtgctggtggtggccaaggtggagaagggcaagagcaagaagctgaagagcgtgaaggagctgctgggcatcaccatcatggagcgcagcagcttcgagaagaaccccatcgacttcctggaggccaagggctacaaggaggtgaagaaggacctgatcatcaagctgcccaagtacagcctgttcgagctggagaacggccgcaagcgcatgctggccagcgccggcgagctgcagaagggcaacgagctggccctgcccagcaagtacgtgaacttcctgtacctggccagccactacgagaagctgaagggcagccccgaggacaacgagcagaagcagctgttcgtggagcagcacaagcactacctggacgagatcatcgagcagatcagcgagttcagcaagcgcgtgatcctggccgacgccaacctggacaaggtgctgagcgcctacaacaagcaccgcgacaagcccatccgcgagcaggccgagaacatcatccacctgttcaccctgaccaacctgggcgcccccgccgccttcaagtacttcgacaccaccatcgaccgcaagcgctacaccagcaccaaggaggtgctggacgccaccctgatccaccagagcatcaccggtctgtacgagacccgcatcgacctgagccagctgggcggcgac

SEQ ID NO: 44 - DNA, 22 bp, synthetic construct
  source 1..22: mol_type = other DNA
aggtgggaaactgaggcttngg

SEQ ID NO: 45 - DNA, 22 bp, synthetic construct
  source 1..22: mol_type = other DNA
acatgcatatgtatgtgtgngg

SEQ ID NO: 46 - DNA, 22 bp, synthetic construct
  source 1..22: mol_type = other DNA
gaatcccttctgcagcaccngg

SEQ ID NO: 47 - DNA, 22 bp, synthetic construct
  source 1..22: mol_type = other DNA
ggtggggggagtttgctccngg

SEQ ID NO: 48 - DNA, 22 bp, synthetic construct
  source 1..22: mol_type = other DNA
ttgccccacagggcagtaangg

SEQ ID NO: 49 - DNA, 22 bp, synthetic construct
  source 1..22: mol_type = other DNA
acttgtgtgtgtgtgtgggggg

SEQ ID NO: 50 - DNA, 22 bp, synthetic construct
  source 1..22: mol_type = other DNA
atatatatatatatatatggag

SEQ ID NO: 51 - DNA, 23 bp, synthetic construct
  source 1..23: mol_type = other DNA
tagatatatatgaatgggtagag

SEQ ID NO: 52 - DNA, 22 bp, synthetic construct
  source 1..22: mol_type = other DNA
aggtgggaaactgaggcccagg

SEQ ID NO: 53 - DNA, 23 bp, synthetic construct
  source 1..23: mol_type = other DNA
tgatgcatatgtatgtgtggagg

SEQ ID NO: 54 - DNA, 22 bp, synthetic construct
  source 1..22: mol_type = other DNA
aaatgcatatgtatgagtgtgg

SEQ ID NO: 55 - DNA, 21 bp, synthetic construct
  source 1..21: mol_type = other DNA
catgcatatgcatgtgggagg

SEQ ID NO: 56 - DNA, 22 bp, synthetic construct
  source 1..22: mol_type = other DNA
agatgcataggtatgtgtgtgg

SEQ ID NO: 57 - DNA, 22 bp, synthetic construct
  source 1..22: mol_type = other DNA
acttgcatatctatgtgtgtgg

SEQ ID NO: 58 - DNA, 22 bp, synthetic construct
  source 1..22: mol_type = other DNA
ccgtgggaaactgaggcttggg

SEQ ID NO: 59 - DNA, 22 bp, synthetic construct
  source 1..22: mol_type = other DNA
aggtgggaaactgaggctgagg

SEQ ID NO: 60 - DNA, 22 bp, synthetic construct
  source 1..22: mol_type = other DNA
aggagggaaactgaggctcagg

SEQ ID NO: 61 - DNA, 22 bp, synthetic construct
  source 1..22: mol_type = other DNA
aaatacatatgtatgtgtgtgg

SEQ ID NO: 62 - DNA, 22 bp, synthetic construct
  source 1..22: mol_type = other DNA
acatgtatatgtatatgtgtgg

SEQ ID NO: 63 - DNA, 22 bp, synthetic construct
  source 1..22: mol_type = other DNA
acatatatatgtatgtgtgtgg

SEQ ID NO: 64 - DNA, 23 bp, synthetic construct
  source 1..23: mol_type = other DNA
gggtgggtggagtttgctactgg

SEQ ID NO: 65 - DNA, 23 bp, synthetic construct
  source 1..23: mol_type = other DNA
aggtggtgggagcttgttcctgg

SEQ ID NO: 66 - DNA, 23 bp, synthetic construct
  source 1..23: mol_type = other DNA
ggtgggggtgggtttgctcctgg

SEQ ID NO: 67 - DNA, 23 bp, synthetic construct
  source 1..23: mol_type = other DNA
gggcaaggggaggttgctcctgg

SEQ ID NO: 68 - DNA, 23 bp, synthetic construct
  source 1..23: mol_type = other DNA
ggattgccatccgcagcacctgg

SEQ ID NO: 69 - DNA, 23 bp, synthetic construct
  source 1..23: mol_type = other DNA
ggagtccctcctgcagcacctga

SEQ ID NO: 70 - DNA, 23 bp, synthetic construct
  source 1..23: mol_type = other DNA
agaggcccctctgcagcaccagg

SEQ ID NO: 71 - DNA, 23 bp, synthetic construct
  source 1..23: mol_type = other DNA
accatccctcctgcagcaccagg

SEQ ID NO: 72 - DNA, 20 bp, synthetic construct
  source 1..20: mol_type = other DNA
gaccccctccaccccgcctc

SEQ ID NO: 73 - DNA, 20 bp, synthetic construct
  source 1..20: mol_type = other DNA
agcagcagcggcggcaacag

SEQ ID NO: 74 - DNA, 19 bp, synthetic construct
  source 1..19: mol_type = other DNA
ggtggggaaactgaggctt

SEQ ID NO: 75 - DNA, 19 bp, synthetic construct
  source 1..19: mol_type = other DNA
gagtgggaaactgaggctt

SEQ ID NO: 76 - DNA, 19 bp, synthetic construct
  source 1..19: mol_type = other DNA
aagtgggagactgaggctt

SEQ ID NO: 77 - DNA, 19 bp, synthetic construct
  source 1..19: mol_type = other DNA
aggtgagaaactgaggctc

SEQ ID NO: 78 - DNA, 19 bp, synthetic construct
  source 1..19: mol_type = other DNA
aggtaggaaactgaagctt

SEQ ID NO: 79 - DNA, 19 bp, synthetic construct
  source 1..19: mol_type = other DNA
agtagtgaaaataaacata

SEQ ID NO: 80 - DNA, 19 bp, synthetic construct
  source 1..19: mol_type = other DNA
agacagaaaactgaggctt

SEQ ID NO: 81 - DNA, 19 bp, synthetic construct
  source 1..19: mol_type = other DNA
aggggagaaactgaggctt

SEQ ID NO: 82 - DNA, 19 bp, synthetic construct
  source 1..19: mol_type = other DNA
aggggagaaactgaggctt

SEQ ID NO: 83 - DNA, 19 bp, synthetic construct
  source 1..19: mol_type = other DNA
gtgtaggaaaccaaggctt

SEQ ID NO: 84 - DNA, 19 bp, synthetic construct
  source 1..19: mol_type = other DNA
tctggggaaactgaggcct

SEQ ID NO: 85 - DNA, 19 bp, synthetic construct
  source 1..19: mol_type = other DNA
agatgagaaactgaggctt

SEQ ID NO: 86 - DNA, 19 bp, synthetic construct
  source 1..19: mol_type = other DNA
agttgggaagatgaggctt

SEQ ID NO: 87 - DNA, 19 bp, synthetic construct
  source 1..19: mol_type = other DNA
aggtgggaaattgaggcat

SEQ ID NO: 88 - DNA, 19 bp, synthetic construct
  source 1..19: mol_type = other DNA
aggtgagcaactgaggctt

SEQ ID NO: 89 - DNA, 19 bp, synthetic construct
  source 1..19: mol_type = other DNA
aggtgggaaactgaggctg

SEQ ID NO: 90 - DNA, 19 bp, synthetic construct
  source 1..19: mol_type = other DNA
aggtaggaagctgaggctt

SEQ ID NO: 91 - DNA, 19 bp, synthetic construct
  source 1..19: mol_type = other DNA
agatgggaaactgaggctt

SEQ ID NO: 92 - DNA, 19 bp, synthetic construct
  source 1..19: mol_type = other DNA
gctggggaaactgaggctt

SEQ ID NO: 93 - DNA, 19 bp, synthetic construct
  source 1..19: mol_type = other DNA
aggtgggaaactgaggctt

SEQ ID NO: 94 - DNA, 19 bp, synthetic construct
  source 1..19: mol_type = other DNA
ggtggggaaactgaggctt

SEQ ID NO: 95 - DNA, 19 bp, synthetic construct
  source 1..19: mol_type = other DNA
aggtgggaaactgaggccc

SEQ ID NO: 96 - DNA, 19 bp, synthetic construct
  source 1..19: mol_type = other DNA
ggatgaaaaactgaggctt

SEQ ID NO: 97 - DNA, 19 bp, synthetic construct
  source 1..19: mol_type = other DNA
gacaaggaaactgaggctc

SEQ ID NO: 98 - DNA, 19 bp, synthetic construct
  source 1..19: mol_type = other DNA
aggtgggaaactgaggcaa

SEQ ID NO: 99 - DNA, 19 bp, synthetic construct
  source 1..19: mol_type = other DNA
agtggggaaactgaggctt

SEQ ID NO: 100 - DNA, 19 bp, synthetic construct
  source 1..19: mol_type = other DNA
aggtggaaaactgaggctt

SEQ ID NO: 101 - DNA, 19 bp, synthetic construct
  source 1..19: mol_type = other DNA
atgtgcctctctaaggctc

SEQ ID NO: 102 - DNA, 19 bp, synthetic construct
  source 1..19: mol_type = other DNA
aaggaggaaactgaggctt

SEQ ID NO: 103 - DNA, 19 bp, synthetic construct
  source 1..19: mol_type = other DNA
agacaggaaactgaggctt

SEQ ID NO: 104 - DNA, 19 bp, synthetic construct
  source 1..19: mol_type = other DNA
cgtcgggaaactgaggctt

SEQ ID NO: 105 - DNA, 19 bp, synthetic construct
  source 1..19: mol_type = other DNA
gagtgggaaactgaggctt

SEQ ID NO: 106 - DNA, 19 bp, synthetic construct
  source 1..19: mol_type = other DNA
ggtggggaaactgaggctt

SEQ ID NO: 107 - DNA, 19 bp, synthetic construct
  source 1..19: mol_type = other DNA
aggcaggaaactgaggctt

SEQ ID NO: 108 - DNA, 19 bp, synthetic construct
  source 1..19: mol_type = other DNA
agataggaaactgaggctt

SEQ ID NO: 109 - DNA, 19 bp, synthetic construct
  source 1..19: mol_type = other DNA
aggtaggaaactgaggctt

SEQ ID NO: 110 - DNA, 19 bp, synthetic construct
  source 1..19: mol_type = other DNA
gattgggaaactgaggctt

SEQ ID NO: 111 - DNA, 19 bp, synthetic construct
  source 1..19: mol_type = other DNA
agtagggaaactgaggctt

SEQ ID NO: 112 - DNA, 19 bp, synthetic construct
  source 1..19: mol_type = other DNA
tatagggaaactgaggctt

SEQ ID NO: 113 - DNA, 19 bp, synthetic construct
  source 1..19: mol_type = other DNA
agggaggaaactgaggctc

SEQ ID NO: 114 - DNA, 19 bp, synthetic construct
  source 1..19: mol_type = other DNA
aggtgggaaactgaggcac

SEQ ID NO: 115 - DNA, 19 bp, synthetic construct
  source 1..19: mol_type = other DNA
gatggggaaactgaggctt

SEQ ID NO: 116 - DNA, 19 bp, synthetic construct
  source 1..19: mol_type = other DNA
agtggggaaactgaggctt

SEQ ID NO: 117 - DNA, 19 bp, synthetic construct
  source 1..19: mol_type = other DNA
gaggaggaaactgaggctt

SEQ ID NO: 118 - DNA, 19 bp, synthetic construct
  source 1..19: mol_type = other DNA
agatgtgaaaatgaggctt

SEQ ID NO: 119 - DNA, 19 bp, synthetic construct
  source 1..19: mol_type = other DNA
gatggggaaactgaggctt

SEQ ID NO: 120 - DNA, 19 bp, synthetic construct
  source 1..19: mol_type = other DNA
aagtaggaaactgaggctt

SEQ ID NO: 121 - DNA, 19 bp, synthetic construct
  source 1..19: mol_type = other DNA
agaggggaaactgaggctt

SEQ ID NO: 122 - DNA, 19 bp, synthetic construct
  source 1..19: mol_type = other DNA
aggtgggaaactgaggctc

SEQ ID NO: 123 - DNA, 19 bp, synthetic construct
  source 1..19: mol_type = other DNA
gatggggaaactgaggctt

SEQ ID NO: 124 - DNA, 19 bp, synthetic construct
  source 1..19: mol_type = other DNA
gatggggaaactgaggctt

SEQ ID NO: 125 - DNA, 19 bp, synthetic construct
  source 1..19: mol_type = other DNA
gaaggggaaactgaggctt

SEQ ID NO: 126 - DNA, 19 bp, synthetic construct
  source 1..19: mol_type = other DNA
agaggggaaactgaggctt

SEQ ID NO: 127 - DNA, 19 bp, synthetic construct
  source 1..19: mol_type = other DNA
aggttggaaactgaggcct

SEQ ID NO: 128 - DNA, 19 bp, synthetic construct
  source 1..19: mol_type = other DNA
aaaagggaaactgaggctt

SEQ ID NO: 129 - DNA, 19 bp, synthetic construct
  source 1..19: mol_type = other DNA
agatggggcaatgaggctt

SEQ ID NO: 130 - DNA, 19 bp, synthetic construct
  source 1..19: mol_type = other DNA
agatgggaaactgaggctt

SEQ ID NO: 131 - DNA, 19 bp, synthetic construct
  source 1..19: mol_type = other DNA
agaggggaaactgaggctt

SEQ ID NO: 132 - DNA, 19 bp, synthetic construct
  source 1..19: mol_type = other DNA
gataaggaaactgaagctt

SEQ ID NO: 133 - DNA, 19 bp, synthetic construct
  source 1..19: mol_type = other DNA
tgatgcatatgtatgtgtg

SEQ ID NO: 134 - DNA, 19 bp, synthetic construct
  source 1..19: mol_type = other DNA
acacgcatgtgtatgtgtg

SEQ ID NO: 135 - DNA, 19 bp, synthetic construct
  source 1..19: mol_type = other DNA
acacgcatatgtatgtgtg

SEQ ID NO: 136 - DNA, 19 bp, synthetic construct
  source 1..19: mol_type = other DNA
tcatgaatatgtgtgtgtg

SEQ ID NO: 137 - DNA, 19 bp, synthetic construct
  source 1..19: mol_type = other DNA
acatacatatgtatatata

SEQ ID NO: 138 - DNA, 19 bp, synthetic construct
  source 1..19: mol_type = other DNA
acacgcatacgtatgtgta

SEQ ID NO: 139 - DNA, 19 bp, synthetic construct
  source 1..19: mol_type = other DNA
tcatacatatgtatgtatg

SEQ ID NO: 140 - DNA, 19 bp, synthetic construct
  source 1..19: mol_type = other DNA
aaatgcatatgtatgggtt

SEQ ID NO: 141 - DNA, 19 bp, synthetic construct
  source 1..19: mol_type = other DNA
catgctgtgtatgtgtgtg

SEQ ID NO: 142 - DNA, 19 bp, synthetic construct
  source 1..19: mol_type = other DNA
acatgcatatggatgtgtg

SEQ ID NO: 143 - DNA, 19 bp, synthetic construct
  source 1..19: mol_type = other DNA
acatgcatatgtatatgtg

SEQ ID NO: 144 - DNA, 19 bp, synthetic construct
  source 1..19: mol_type = other DNA
aaatgcatatgtatgagtg

SEQ ID NO: 145 - DNA, 19 bp, synthetic construct
  source 1..19: mol_type = other DNA
gcatacatatgtatgtata

SEQ ID NO: 146 - DNA, 19 bp, synthetic construct
  source 1..19: mol_type = other DNA
tcatgcatatgcatgtggg

SEQ ID NO: 147 - DNA, 19 bp, synthetic construct
  source 1..19: mol_type = other DNA
acacacatatgtatatgta

SEQ ID NO: 148 - DNA, 19 bp, synthetic construct
  source 1..19: mol_type = other DNA
gcatgtgtatgtatgtgtg

SEQ ID NO: 149 - DNA, 19 bp, synthetic construct
  source 1..19: mol_type = other DNA
acatgcatatatatgtgta

SEQ ID NO: 150 - DNA, 19 bp, synthetic construct
  source 1..19: mol_type = other DNA
agatgaatatgtgtgtgtg

SEQ ID NO: 151 - DNA, 19 bp, synthetic construct
  source 1..19: mol_type = other DNA
acatgcatatgtatgtatg

SEQ ID NO: 152 - DNA, 19 bp, synthetic construct
  source 1..19: mol_type = other DNA
acatacacatgtatgtgta

SEQ ID NO: 153 - DNA, 19 bp, synthetic construct
  source 1..19: mol_type = other DNA
acacacatatatatgtgta

SEQ ID NO: 154 - DNA, 19 bp, synthetic construct
  source 1..19: mol_type = other DNA
agatgcataggtatgtgtg

SEQ ID NO: 155 - DNA, 19 bp, synthetic construct
  source 1..19: mol_type = other DNA
acatacatatatatatgta

SEQ ID NO: 156 - DNA, 19 bp, synthetic construct
  source 1..19: mol_type = other DNA
acatgcatacatatgtgtg

SEQ ID NO: 157 - DNA, 19 bp, synthetic construct
  source 1..19: mol_type = other DNA
acatgtatatatatgtata

SEQ ID NO: 158 - DNA, 19 bp, synthetic construct
  source 1..19: mol_type = other DNA
acatgcatatctatgtgtg

SEQ ID NO: 159 - DNA, 19 bp, synthetic construct
  source 1..19: mol_type = other DNA
aaatgcatatatatgtata

SEQ ID NO: 160 - DNA, 19 bp, synthetic construct
  source 1..19: mol_type = other DNA
acttgcatatctatgtgtg

SEQ ID NO: 161 - DNA, 19 bp, synthetic construct
  source 1..19: mol_type = other DNA
aaatgcatatgtatgtgtg

SEQ ID NO: 162 - DNA, 19 bp, synthetic construct
  source 1..19: mol_type = other DNA
acatgtatatgtatatata

SEQ ID NO: 163 - DNA, 19 bp, synthetic construct
  source 1..19: mol_type = other DNA
acacacatatatatgtgtg

SEQ ID NO: 164 - DNA, 19 bp, synthetic construct
  source 1..19: mol_type = other DNA
acatacatatgtatgtgtg

SEQ ID NO: 165 - DNA, 19 bp, synthetic construct
  source 1..19: mol_type = other DNA
acatgcatatgtatgtgtg

SEQ ID NO: 166 - DNA, 19 bp, synthetic construct
  source 1..19: mol_type = other DNA
gcatgcataggtatgtgtg

SEQ ID NO: 167 - DNA, 19 bp, synthetic construct
  source 1..19: mol_type = other DNA
acatgcatgtgtatgtgtg

SEQ ID NO: 168 - DNA, 19 bp, synthetic construct
  source 1..19: mol_type = other DNA
acatgcatatgtacgtgta

SEQ ID NO: 169 - DNA, 19 bp, synthetic construct
  source 1..19: mol_type = other DNA
agatgcatatgtatatatg

SEQ ID NO: 170 - DNA, 19 bp, synthetic construct
  source 1..19: mol_type = other DNA
ccatgcatatgtatatatg

SEQ ID NO: 171 - DNA, 19 bp, synthetic construct
  source 1..19: mol_type = other DNA
atatgcatatatatgtgtg

SEQ ID NO: 172 - DNA, 19 bp, synthetic construct
  source 1..19: mol_type = other DNA
gcatgcaaatgaatgtgtg

SEQ ID NO: 173 - DNA, 19 bp, synthetic construct
  source 1..19: mol_type = other DNA
atatgcatatgtatgtgta

SEQ ID NO: 174 - DNA, 19 bp, synthetic construct
  source 1..19: mol_type = other DNA
tcatgcatatgtatgtgga

SEQ ID NO: 175 - DNA, 19 bp, synthetic construct
  source 1..19: mol_type = other DNA
agatagaaaactaagactt

SEQ ID NO: 176 - DNA, 19 bp, synthetic construct
  source 1..19: mol_type = other DNA
gattgggaaactgaggctt

SEQ ID NO: 177 - DNA, 19 bp, synthetic construct
  source 1..19: mol_type = other DNA
aggtgggaaactgaggctt

SEQ ID NO: 178 - DNA, 19 bp, synthetic construct
  source 1..19: mol_type = other DNA
gaaggggaaactgaggctt

SEQ ID NO: 179 - DNA, 19 bp, synthetic construct
  source 1..19: mol_type = other DNA
aggcaggaaactggagctt

SEQ ID NO: 180 - DNA, 19 bp, synthetic construct
  source 1..19: mol_type = other DNA
agatgggaaactgaggctt

SEQ ID NO: 181 - DNA, 19 bp, synthetic construct
  source 1..19: mol_type = other DNA
acgtgggaaactgaggcct

SEQ ID NO: 182 - DNA, 19 bp, synthetic construct
  source 1..19: mol_type = other DNA
ccgtgggaaactgaggctt

SEQ ID NO: 183 - DNA, 19 bp, synthetic construct
  source 1..19: mol_type = other DNA
aggggggaaactgaggcat

SEQ ID NO: 184 - DNA, 19 bp, synthetic construct
  source 1..19: mol_type = other DNA
agctgggaaactgaggctt

SEQ ID NO: 185 - DNA, 19 bp, synthetic construct
  source 1..19: mol_type = other DNA
gaggaggaaactgaggctt

SEQ ID NO: 186 - DNA, 19 bp, synthetic construct
  source 1..19: mol_type = other DNA
tggtgggaaacagaggctt

SEQ ID NO: 187 - DNA, 19 bp, synthetic construct
  source 1..19: mol_type = other DNA
agacaggaaactgaggctt

SEQ ID NO: 188 - DNA, 19 bp, synthetic construct
  source 1..19: mol_type = other DNA
ggagaggaaactgaggctt

SEQ ID NO: 189 - DNA, 19 bp, synthetic construct
  source 1..19: mol_type = other DNA
cctggggaaactgaggctt

SEQ ID NO: 190 - DNA, 19 bp, synthetic construct
  source 1..19: mol_type = other DNA
gctggggaaactgaggctt

SEQ ID NO: 191 - DNA, 19 bp, synthetic construct
  source 1..19: mol_type = other DNA
gccagggaaactgaggctt

SEQ ID NO: 192 - DNA, 19 bp, synthetic construct
  source 1..19: mol_type = other DNA
gaggaggaaactgaggctt

SEQ ID NO: 193 - DNA, 19 bp, synthetic construct
  source 1..19: mol_type = other DNA
aagtggtaaactgaggctt

SEQ ID NO: 194 - DNA, 19 bp, synthetic construct
  source 1..19: mol_type = other DNA
aactgggaaactgaggctt

SEQ ID NO: 195 - DNA, 19 bp, synthetic construct
  source 1..19: mol_type = other DNA
aggagagaaactgaggctt

SEQ ID NO: 196 - DNA, 19 bp, synthetic construct
  source 1..19: mol_type = other DNA
aaacaagaaactgaagctt

SEQ ID NO: 197 - DNA, 19 bp, synthetic construct
  source 1..19: mol_type = other DNA
caggaggaaactgaggctt

SEQ ID NO: 198 - DNA, 19 bp, synthetic construct
  source 1..19: mol_type = other DNA
aggtgggaaactgagaccc

SEQ ID NO: 199 - DNA, 19 bp, synthetic construct
  source 1..19: mol_type = other DNA
agacagaaaactgagactt

SEQ ID NO: 200 - DNA, 19 bp, synthetic construct
  source 1..19: mol_type = other DNA
agaggggaaactgaggctt

SEQ ID NO: 201 - DNA, 19 bp, synthetic construct
  source 1..19: mol_type = other DNA
aggtgggaaactgaggctg

SEQ ID NO: 202 - DNA, 19 bp, synthetic construct
  source 1..19: mol_type = other DNA
tatggggaaactgaggctt

SEQ ID NO: 203 - DNA, 19 bp, synthetic construct
  source 1..19: mol_type = other DNA
gggggggaaactggggctt

SEQ ID NO: 204 - DNA, 19 bp, synthetic construct
  source 1..19: mol_type = other DNA
tggagggaaactgaggctt

SEQ ID NO: 205 - DNA, 19 bp, synthetic construct
  source 1..19: mol_type = other DNA
aggtgggaaactgaggctt

SEQ ID NO: 206 - DNA, 19 bp, synthetic construct
  source 1..19: mol_type = other DNA
agccgggaaactgaggctt

SEQ ID NO: 207 - DNA, 19 bp, synthetic construct
  source 1..19: mol_type = other DNA
ggtgggaagactgaggctt

SEQ ID NO: 208 - DNA, 19 bp, synthetic construct
  source 1..19: mol_type = other DNA
aggagggaaactgaggctc

SEQ ID NO: 209 - DNA, 19 bp, synthetic construct
  source 1..19: mol_type = other DNA
tggtgggaaactgaggctt

SEQ ID NO: 210 - DNA, 19 bp, synthetic construct
  source 1..19: mol_type = other DNA
agatgaaaaactgaggctt

SEQ ID NO: 211 - DNA, 19 bp, synthetic construct
  source 1..19: mol_type = other DNA
aggagggaaactgaggctt

SEQ ID NO: 212 - DNA, 19 bp, synthetic construct
  source 1..19: mol_type = other DNA
ttttgcatatgtatgtgtg

SEQ ID NO: 213 - DNA, 19 bp, synthetic construct
  source 1..19: mol_type = other DNA
acatgcatatgtatatgta

SEQ ID NO: 214 - DNA, 19 bp, synthetic construct
  source 1..19: mol_type = other DNA
atatgcatatgtatatgtg

SEQ ID NO: 215 - DNA, 19 bp, synthetic construct
  source 1..19: mol_type = other DNA
gcatgaatgtgtatgtgtg

SEQ ID NO: 216 - DNA, 19 bp, synthetic construct
  source 1..19: mol_type = other DNA
acacgcatatgtatgtgtg

SEQ ID NO: 217 - DNA, 19 bp, synthetic construct
  source 1..19: mol_type = other DNA
acatacacatatatatgta

SEQ ID NO: 218 - DNA, 19 bp, synthetic construct
  source 1..19: mol_type = other DNA
acatgcatatgtatgtgtg

SEQ ID NO: 219 - DNA, 19 bp, synthetic construct
  source 1..19: mol_type = other DNA
acatgcacatgcatgtgtg

SEQ ID NO: 220 - DNA, 19 bp, synthetic construct
  source 1..19: mol_type = other DNA
taatgcatatgtatgtgtg

SEQ ID NO: 221 - DNA, 19 bp, synthetic construct
  source 1..19: mol_type = other DNA
tgatgcatatgtatgtgtg

SEQ ID NO: 222 - DNA, 19 bp, synthetic construct
  source 1..19: mol_type = other DNA
gcatgcgtgtgtatgtgtg

SEQ ID NO: 223 - DNA, 19 bp, synthetic construct
  source 1..19: mol_type = other DNA
acatacatatatatatgtg

SEQ ID NO: 224 - DNA, 19 bp, synthetic construct
  source 1..19: mol_type = other DNA
acatgcatatgtatgtgtg

SEQ ID NO: 225 - DNA, 19 bp, synthetic construct
  source 1..19: mol_type = other DNA
atatacgtgtgtatctctg

SEQ ID NO: 226 - DNA, 19 bp, synthetic construct
  source 1..19: mol_type = other DNA
tcatgaataggtatgtggg

SEQ ID NO: 227 - DNA, 19 bp, synthetic construct
  source 1..19: mol_type = other DNA
acacacacatatatgtgtg

SEQ ID NO: 228 - DNA, 19 bp, synthetic construct
  source 1..19: mol_type = other DNA
acaagtatatgtatgtaag

SEQ ID NO: 229 - DNA, 19 bp, synthetic construct
  source 1..19: mol_type = other DNA
acatgcatatgtatgtgtg

SEQ ID NO: 230 - DNA, 19 bp, synthetic construct
  source 1..19: mol_type = other DNA
aaatacatatgtatgtgtg

SEQ ID NO: 231 - DNA, 19 bp, synthetic construct
  source 1..19: mol_type = other DNA
acatgcatatgtatatatg

SEQ ID NO: 232 - DNA, 19 bp, synthetic construct
  source 1..19: mol_type = other DNA
acatgcatatgtgtgtgtg

SEQ ID NO: 233 - DNA, 19 bp, synthetic construct
  source 1..19: mol_type = other DNA
acatgtatatgtatatgtg

SEQ ID NO: 234 - DNA, 19 bp, synthetic construct
  source 1..19: mol_type = other DNA
gcatgcatatgcatgtgtg

SEQ ID NO: 235 - DNA, 19 bp, synthetic construct
  source 1..19: mol_type = other DNA
gtatatgtatgtatgtgtg

SEQ ID NO: 236 - DNA, 19 bp, synthetic construct
  source 1..19: mol_type = other DNA
acatgcatatgaatgagtg

SEQ ID NO: 237 - DNA, 19 bp, synthetic construct
  source 1..19: mol_type = other DNA
gtgtgcatatgtatgtgtg

SEQ ID NO: 238 - DNA, 19 bp, synthetic construct
  source 1..19: mol_type = other DNA
acatatatatgtatgtgtg

SEQ ID NO: 239 - DNA, 19 bp, synthetic construct
  source 1..19: mol_type = other DNA
gtgtgcatatgtatgtgtg

SEQ ID NO: 240 - DNA, 19 bp, synthetic construct
  source 1..19: mol_type = other DNA
gtatgcatatgtatgtatg

SEQ ID NO: 241 - DNA, 19 bp, synthetic construct
  source 1..19: mol_type = other DNA
gtatgcatatgtatatgtg

SEQ ID NO: 242 - DNA, 19 bp, synthetic construct
  source 1..19: mol_type = other DNA
acatgcatatgtatgtgca

SEQ ID NO: 243 - DNA, 19 bp, synthetic construct
  source 1..19: mol_type = other DNA
acctgcatatgtatgtgtg

SEQ ID NO: 244 - DNA, 19 bp, synthetic construct
  source 1..19: mol_type = other DNA
acatgagtatgtatgtgag

SEQ ID NO: 245 - DNA, 19 bp, synthetic construct
  source 1..19: mol_type = other DNA
acacgcatatgtgtgtgag

SEQ ID NO: 246 - DNA, 19 bp, synthetic construct
  source 1..19: mol_type = other DNA
gtatgcatatatatgtgtg

SEQ ID NO: 247 - DNA, 19 bp, synthetic construct
  source 1..19: mol_type = other DNA
acatgcataggtatgtgtg

SEQ ID NO: 248 - DNA, 19 bp, synthetic construct
  source 1..19: mol_type = other DNA
acatgcatatgtatgtatg

SEQ ID NO: 249 - DNA, 19 bp, synthetic construct
  source 1..19: mol_type = other DNA
acatgcatatgtatgtgtg

SEQ ID NO: 250 - DNA, 19 bp, synthetic construct
  source 1..19: mol_type = other DNA
gtccccacagggtcagtaa

SEQ ID NO: 251 - DNA, 19 bp, synthetic construct
  source 1..19: mol_type = other DNA
ctaccccacatggcagtaa

SEQ ID NO: 252 - DNA, 19 bp, synthetic construct
  source 1..19: mol_type = other DNA
ctgcccagtaaggcagtaa

SEQ ID NO: 253 - DNA, 19 bp, synthetic construct
  source 1..19: mol_type = other DNA
tgtccccacagggcaggaa

SEQ ID NO: 254 - DNA, 19 bp, synthetic construct
  source 1..19: mol_type = other DNA
cagccccacagggcactag

SEQ ID NO: 255 - DNA, 19 bp, synthetic construct
  source 1..19: mol_type = other DNA
ctaccccacagggcattag

SEQ ID NO: 256 - DNA, 19 bp, synthetic construct
  source 1..19: mol_type = other DNA
tagccccacagggcaggtt

SEQ ID NO: 257 - DNA, 19 bp, synthetic construct
  source 1..19: mol_type = other DNA
ttacctcacagagcagaaa

SEQ ID NO: 258 - DNA, 19 bp, synthetic construct
  source 1..19: mol_type = other DNA
ataccccacaggtcagtaa

SEQ ID NO: 259 - DNA, 19 bp, synthetic construct
  source 1..19: mol_type = other DNA
ctgccccacaggccaggaa

SEQ ID NO: 260 - DNA, 19 bp, synthetic construct
  source 1..19: mol_type = other DNA
aagccctacagggcagcaa

SEQ ID NO: 261 - DNA, 19 bp, synthetic construct
  source 1..19: mol_type = other DNA
cctccccacagggcagtca

SEQ ID NO: 262 - DNA, 19 bp, synthetic construct
  source 1..19: mol_type = other DNA
gtgccacacacagcagtaa

SEQ ID NO: 263 - DNA, 19 bp, synthetic construct
  source 1..19: mol_type = other DNA
cagccccacaggtcagcaa

SEQ ID NO: 264 - DNA, 19 bp, synthetic construct
  source 1..19: mol_type = other DNA
cagccccaccgggcagtag

SEQ ID NO: 265 - DNA, 19 bp, synthetic construct
  source 1..19: mol_type = other DNA
cagccccacagggcataaa

SEQ ID NO: 266 - DNA, 19 bp, synthetic construct
  source 1..19: mol_type = other DNA
cagccccacagggcagtaa

SEQ ID NO: 267 - DNA, 19 bp, synthetic construct
  source 1..19: mol_type = other DNA
ttgcccctcagggcagcta

SEQ ID NO: 268 - DNA, 19 bp, synthetic construct
  source 1..19: mol_type = other DNA
ctgccccacagggcaatta

SEQ ID NO: 269 - DNA, 19 bp, synthetic construct
  source 1..19: mol_type = other DNA
aagccccacagggcagaca

SEQ ID NO: 270 - DNA, 19 bp, synthetic construct
  source 1..19: mol_type = other DNA
aggccccacaggacaggaa

SEQ ID NO: 271 - DNA, 19 bp, synthetic construct
  source 1..19: mol_type = other DNA
ttgccccacagggcagtaa

SEQ ID NO: 272 - DNA, 19 bp, synthetic construct
  source 1..19: mol_type = other DNA
tgcccctcagggacagtat

SEQ ID NO: 273 - DNA, 19 bp, synthetic construct
  source 1..19: mol_type = other DNA
atgcctcacaggacaggaa

SEQ ID NO: 274 - DNA, 19 bp, synthetic construct
  source 1..19: mol_type = other DNA
aggccccgcagggcagttt

SEQ ID NO: 275 - DNA, 19 bp, synthetic construct
  source 1..19: mol_type = other DNA
ttgccccacggggcagtga

SEQ ID NO: 276 - DNA, 19 bp, synthetic construct
  source 1..19: mol_type = other DNA
ctgccccacagggcagcaa

SEQ ID NO: 277 - DNA, 19 bp, synthetic construct
  source 1..19: mol_type = other DNA
gagccccacagggcagaga

SEQ ID NO: 278 - DNA, 19 bp, synthetic construct
  source 1..19: mol_type = other DNA
ttatcccacaggacagtga

SEQ ID NO: 279 - DNA, 19 bp, synthetic construct
  source 1..19: mol_type = other DNA
tggccccacaaggcagaaa

SEQ ID NO: 280 - DNA, 19 bp, synthetic construct
  source 1..19: mol_type = other DNA
cagccccacagggcagtaa

SEQ ID NO: 281 - DNA, 19 bp, synthetic construct
  source 1..19: mol_type = other DNA
ttaccacacagagcagtta

SEQ ID NO: 282 - DNA, 19 bp, synthetic construct
  source 1..19: mol_type = other DNA
ttgcccctcaggacagtac

SEQ ID NO: 283 - DNA, 19 bp, synthetic construct
  source 1..19: mol_type = other DNA
cagccccacaggtcagtga

SEQ ID NO: 284 - DNA, 19 bp, synthetic construct
  source 1..19: mol_type = other DNA
tgctcccacagggcagtaa

SEQ ID NO: 285 - DNA, 19 bp, synthetic construct
  source 1..19: mol_type = other DNA
ctctcccacagggcagtaa

SEQ ID NO: 286 - DNA, 19 bp, synthetic construct
  source 1..19: mol_type = other DNA
attacccccagggcaggaa

SEQ ID NO: 287 - DNA, 19 bp, synthetic construct
  source 1..19: mol_type = other DNA
aatccccacagggcagtaa

SEQ ID NO: 288 - DNA, 19 bp, synthetic construct
  source 1..19: mol_type = other DNA
ctgctccacagggcaggta

SEQ ID NO: 289 - DNA, 19 bp, synthetic construct
  source 1..19: mol_type = other DNA
ttgccccccaggtcagtag

SEQ ID NO: 290 - DNA, 19 bp, synthetic construct
  source 1..19: mol_type = other DNA
gtggcccccagggcagtga

SEQ ID NO: 291 - DNA, 19 bp, synthetic construct
  source 1..19: mol_type = other DNA
gtgccccacagagcactaa

SEQ ID NO: 292 - DNA, 19 bp, synthetic construct
  source 1..19: mol_type = other DNA
gtgccccacaggggagaaa

SEQ ID NO: 293 - DNA, 19 bp, synthetic construct
  source 1..19: mol_type = other DNA
tggccccacagggcaggaa

SEQ ID NO: 294 - DNA, 19 bp, synthetic construct
  source 1..19: mol_type = other DNA
ggtgggtggagtttgctac

SEQ ID NO: 295 - DNA, 19 bp, synthetic construct
  source 1..19: mol_type = other DNA
gggaggggaagtttgctcc

SEQ ID NO: 296 - DNA, 19 bp, synthetic construct
  source 1..19: mol_type = other DNA
gaggaggggagtctgctcc

SEQ ID NO: 297 - DNA, 19 bp, synthetic construct
  source 1..19: mol_type = other DNA
ggtggggagagtttcttcc

SEQ ID NO: 298 - DNA, 19 bp, synthetic construct
  source 1..19: mol_type = other DNA
cctgagggcagtttgctcc

SEQ ID NO: 299 - DNA, 19 bp, synthetic construct
  source 1..19: mol_type = other DNA
gggagggagaatttgctcc

SEQ ID NO: 300 - DNA, 19 bp, synthetic construct
  source 1..19: mol_type = other DNA
ggaaggaggagttagctcc

SEQ ID NO: 301 - DNA, 19 bp, synthetic construct
  source 1..19: mol_type = other DNA
ggtggtgggagcttgttcc

SEQ ID NO: 302 - DNA, 19 bp, synthetic construct
  source 1..19: mol_type = other DNA
gtgggggagagctagctcc

SEQ ID NO: 303 - DNA, 19 bp, synthetic construct
  source 1..19: mol_type = other DNA
agtgggtggagtttgctac

SEQ ID NO: 304 - DNA, 19 bp, synthetic construct
  source 1..19: mol_type = other DNA
agggtggggagtttactcc

SEQ ID NO: 305 - DNA, 19 bp, synthetic construct
  source 1..19: mol_type = other DNA
cgtggggggtgtttgctcc

SEQ ID NO: 306 - DNA, 19 bp, synthetic construct
  source 1..19: mol_type = other DNA
gtgggggtgggtttgctcc

SEQ ID NO: 307 - DNA, 19 bp, synthetic construct
  source 1..19: mol_type = other DNA
ggagcagggaatttgctcc

SEQ ID NO: 308 - DNA, 19 bp, synthetic construct
  source 1..19: mol_type = other DNA
tgggggggcagtttgctcc

SEQ ID NO: 309 - DNA, 19 bp, synthetic construct
  source 1..19: mol_type = other DNA
tgggggtagagtttgctcc

SEQ ID NO: 310 - DNA, 19 bp, synthetic construct
  source 1..19: mol_type = other DNA
ggtggggggagtttgctcc

SEQ ID NO: 311 - DNA, 19 bp, synthetic construct
  source 1..19: mol_type = other DNA
tgtgtggggaatttgctcc

SEQ ID NO: 312 - DNA, 19 bp, synthetic construct
  source 1..19: mol_type = other DNA
caactggggagtttgctcc

SEQ ID NO: 313 - DNA, 19 bp, synthetic construct
  source 1..19: mol_type = other DNA
gggtggggccgtttgctcc

SEQ ID NO: 314 - DNA, 19 bp, synthetic construct
  source 1..19: mol_type = other DNA
ggaggagagagtttgctct

SEQ ID NO: 315 - DNA, 19 bp, synthetic construct
  source 1..19: mol_type = other DNA
agtgggaggagactgctcc

SEQ ID NO: 316 - DNA, 19 bp, synthetic construct
  source 1..19: mol_type = other DNA
ggggtggggagcatgctcc

SEQ ID NO: 317 - DNA, 19 bp, synthetic construct
  source 1..19: mol_type = other DNA
gctggagggagtttgcccc

SEQ ID NO: 318 - DNA, 19 bp, synthetic construct
  source 1..19: mol_type = other DNA
ggcaaggggaggttgctcc

SEQ ID NO: 319 - DNA, 19 bp, synthetic construct
  source 1..19: mol_type = other DNA
ggaaggaggagttagctcc

SEQ ID NO: 320 - DNA, 19 bp, synthetic construct
  source 1..19: mol_type = other DNA
ggaaggaggagttagctcc

SEQ ID NO: 321 - DNA, 19 bp, synthetic construct
  source 1..19: mol_type = other DNA
ggaaggaggagttagctcc

SEQ ID NO: 322 - DNA, 19 bp, synthetic construct
  source 1..19: mol_type = other DNA
ggagggtggagtttgctcc

SEQ ID NO: 323 - DNA, 19 bp, synthetic construct
  source 1..19: mol_type = other DNA
gggggagggagtttgctcc

SEQ ID NO: 324 - DNA, 19 bp, synthetic construct
  source 1..19: mol_type = other DNA
gtttgggggagtttgcccc

SEQ ID NO: 325 - DNA, 19 bp, synthetic construct
  source 1..19: mol_type = other DNA
gttgaggggagtctgctcc

SEQ ID NO: 326 - DNA, 19 bp, synthetic construct
  source 1..19: mol_type = other DNA
tgaggagggagtttgcacc

SEQ ID NO: 327 - DNA, 19 bp, synthetic construct
  source 1..19: mol_type = other DNA
gtagagggagttttgctcc

SEQ ID NO: 328 - DNA, 19 bp, synthetic construct
  source 1..19: mol_type = other DNA
gatggagggagtttgctcc

SEQ ID NO: 329 - DNA, 19 bp, synthetic construct
  source 1..19: mol_type = other DNA
ggggagggaagtttcctcc

SEQ ID NO: 330 - DNA, 19 bp, synthetic construct
  source 1..19: mol_type = other DNA
agtaagggaagtttgctcc

SEQ ID NO: 331 - DNA, 19 bp, synthetic construct
  source 1..19: mol_type = other DNA
ggggtggggactttgctcc

SEQ ID NO: 332 - DNA, 19 bp, synthetic construct
  source 1..19: mol_type = other DNA
agtggagggagcttgctcc

SEQ ID NO: 333 - DNA, 19 bp, synthetic construct
  source 1..19: mol_type = other DNA
tggtgggggagcttgctcc

SEQ ID NO: 334 - DNA, 19 bp, synthetic construct
  source 1..19: mol_type = other DNA
gggaggaggaatttgctcc

SEQ ID NO: 335 - DNA, 19 bp, synthetic construct
  source 1..19: mol_type = other DNA
agtgggaagagtttgttcc

SEQ ID NO: 336 - DNA, 19 bp, synthetic construct
  source 1..19: mol_type = other DNA
gaaaggaggagcttgctcc

SEQ ID NO: 337 - DNA, 19 bp, synthetic construct
  source 1..19: mol_type = other DNA
agggggagcagtttgctcc

SEQ ID NO: 338 - DNA, 19 bp, synthetic construct
  source 1..19: mol_type = other DNA
ggtggggggagtttgcccc

SEQ ID NO: 339 - DNA, 19 bp, synthetic construct
  source 1..19: mol_type = other DNA
ggtcgggggagttagatcc

SEQ ID NO: 340 - DNA, 19 bp, synthetic construct
  source 1..19: mol_type = other DNA
gtgcaggggagcttgctcc

SEQ ID NO: 341 - DNA, 19 bp, synthetic construct
  source 1..19: mol_type = other DNA
ggaggggagagtttgttcc

SEQ ID NO: 342 - DNA, 19 bp, synthetic construct
  source 1..19: mol_type = other DNA
gagggggagagtttgcccc

SEQ ID NO: 343 - DNA, 19 bp, synthetic construct
  source 1..19: mol_type = other DNA
ggtgggagtagttccctgc

SEQ ID NO: 344 - DNA, 19 bp, synthetic construct
  source 1..19: mol_type = other DNA
gcatcccttctgcagccgc

SEQ ID NO: 345 - DNA, 19 bp, synthetic construct
  source 1..19: mol_type = other DNA
gcttccccactgcagcacc

SEQ ID NO: 346 - DNA, 20 bp, synthetic construct
  source 1..20: mol_type = other DNA
gaaccccttctacagcacct

SEQ ID NO: 347 - DNA, 19 bp, synthetic construct
  source 1..19: mol_type = other DNA
tcctttcttctgcagcacc

SEQ ID NO: 348 - DNA, 19 bp, synthetic construct
  source 1..19: mol_type = other DNA
ggaatccctccccagcacc

SEQ ID NO: 349 - DNA, 19 bp, synthetic construct
  source 1..19: mol_type = other DNA
ccctcccttctgcaggcac

SEQ ID NO: 350 - DNA, 19 bp, synthetic construct
  source 1..19: mol_type = other DNA
gaatcctaactgcagcacc

SEQ ID NO: 351 - DNA, 19 bp, synthetic construct
  source 1..19: mol_type = other DNA
atattccctctgcagcacc

SEQ ID NO: 352 - DNA, 19 bp, synthetic construct
  source 1..19: mol_type = other DNA
gattgccatccgcagcacc

SEQ ID NO: 353 - DNA, 19 bp, synthetic construct
  source 1..19: mol_type = other DNA
gtccctcctccgcagcacc

SEQ ID NO: 354 - DNA, 19 bp, synthetic construct
  source 1..19: mol_type = other DNA
gttccccatctgcagcacc

SEQ ID NO: 355 - DNA, 19 bp, synthetic construct
  source 1..19: mol_type = other DNA
tctgtccttctgcagcacc

SEQ ID NO: 356 - DNA, 19 bp, synthetic construct
  source 1..19: mol_type = other DNA
gagtccctcctacagcacc

SEQ ID NO: 357 - DNA, 19 bp, synthetic construct
  source 1..19: mol_type = other DNA
gagtccctcctacagcacc

SEQ ID NO: 358 - DNA, 19 bp, synthetic construct
  source 1..19: mol_type = other DNA
gaatcccatctccagcacc

SEQ ID NO: 359 - DNA, 19 bp, synthetic construct
  source 1..19: mol_type = other DNA
gaatcccttctgcagcacc

SEQ ID NO: 360 - DNA, 19 bp, synthetic construct
  source 1..19: mol_type = other DNA
gaatcccttctacagcatc

SEQ ID NO: 361 - DNA, 19 bp, synthetic construct
  source 1..19: mol_type = other DNA
gaacaccttctgcagctcc

SEQ ID NO: 362 - DNA, 19 bp, synthetic construct
  source 1..19: mol_type = other DNA
cactcccttctgcagcacc

SEQ ID NO: 363 - DNA, 19 bp, synthetic construct
  source 1..19: mol_type = other DNA
gggtcccttctgcagcccc

SEQ ID NO: 364 - DNA, 19 bp, synthetic construct
  source 1..19: mol_type = other DNA
aaataccttctgcagtacc

SEQ ID NO: 365 - DNA, 19 bp, synthetic construct
  source 1..19: mol_type = other DNA
ggaacccttccgcagcacc

SEQ ID NO: 366 - DNA, 19 bp, synthetic construct
  source 1..19: mol_type = other DNA
caaatccttcagcagagcc

SEQ ID NO: 367 - DNA, 19 bp, synthetic construct
  source 1..19: mol_type = other DNA
gcttcccttctgcagcccc

SEQ ID NO: 368 - DNA, 19 bp, synthetic construct
  source 1..19: mol_type = other DNA
gagtccctcctgcagcacc

SEQ ID NO: 369 - DNA, 19 bp, synthetic construct
  source 1..19: mol_type = other DNA
gaaccccctctgcagcttc

SEQ ID NO: 370 - DNA, 19 bp, synthetic construct
  source 1..19: mol_type = other DNA
ctgctgcttctgcagcacc

SEQ ID NO: 371 - DNA, 19 bp, synthetic construct
  source 1..19: mol_type = other DNA
ggtccgcttctgcagcacc

SEQ ID NO: 372 - DNA, 19 bp, synthetic construct
  source 1..19: mol_type = other DNA
ggagtccatctgcagcacc

SEQ ID NO: 373 - DNA, 19 bp, synthetic construct
  source 1..19: mol_type = other DNA
ttcccccttctgcagcccc

SEQ ID NO: 374 - DNA, 19 bp, synthetic construct
  source 1..19: mol_type = other DNA
gaggcccctctgcagcacc

SEQ ID NO: 375 - DNA, 19 bp, synthetic construct
  source 1..19: mol_type = other DNA
gaaccccgtctgcagcacc

SEQ ID NO: 376 - DNA, 19 bp, synthetic construct
  source 1..19: mol_type = other DNA
gtaaggcttctgcagcacc

SEQ ID NO: 377 - DNA, 19 bp, synthetic construct
  source 1..19: mol_type = other DNA
ctgtcccttctgcagctcc

SEQ ID NO: 378 - DNA, 19 bp, synthetic construct
  source 1..19: mol_type = other DNA
ccatccctactgccagcac

SEQ ID NO: 379 - DNA, 19 bp, synthetic construct
  source 1..19: mol_type = other DNA
acatcccttctgcagctcc

SEQ ID NO: 380 - DNA, 19 bp, synthetic construct
  source 1..19: mol_type = other DNA
cgtccccttctgcagcacc

SEQ ID NO: 381 - DNA, 19 bp, synthetic construct
  source 1..19: mol_type = other DNA
ccctccctcctgcagcacc

SEQ ID NO: 382 - DNA, 19 bp, synthetic construct
  source 1..19: mol_type = other DNA
ccatccctcctgcagcacc

SEQ ID NO: 383 - DNA, 19 bp, synthetic construct
  source 1..19: mol_type = other DNA
cactcccttctgcagcacc